European Patent Specification EP 3 930 847 B1, published February 14, 2024. Title: High-Affinity Anti-MERTK Antibodies and Uses Thereof. Applicant: RGENIX, INC. The sequence listing filed with the application follows.

SEQUENCE LISTING (132 sequences)

SEQ ID NO: 1 - protein, 5 aa, Artificial Sequence
  Antibody z10/z11/z13/xAb VH CDR1 (Kabat)
NYGMN

SEQ ID NO: 2 - protein, 7 aa, Artificial Sequence
  Antibody z10/z11/z13/xAb VH CDR1 (Chothia)
GYTFTNY

SEQ ID NO: 3 - protein, 10 aa, Artificial Sequence
  Antibody z10/z11/z13/xAb VH CDR1 (AbM/Exemplary)
GYTFTNYGMN

SEQ ID NO: 4 - protein, 6 aa, Artificial Sequence
  Antibody z10/z11/z13/xAb VH CDR1 (Contact)
TNYGMN

SEQ ID NO: 5 - protein, 8 aa, Artificial Sequence
  Antibody z10/z11/z13/xAb VH CDR1 (IMGT)
GYTFTNYG

SEQ ID NO: 6 - protein, 17 aa, Artificial Sequence
  Antibody z10/z11/z13/xAb VH CDR2 (Kabat/Exemplary)
WINTYTGEPTYADDFKG

SEQ ID NO: 7 - protein, 4 aa, Artificial Sequence
  Antibody z10/z11/z13/xAb VH CDR2 (Chothia)
TYTG

SEQ ID NO: 8 - protein, 10 aa, Artificial Sequence
  Antibody z10/z11/z13/xAb VH CDR2 (AbM)
WINTYTGEPT

SEQ ID NO: 9 - protein, 13 aa, Artificial Sequence
  Antibody z10/z11/z13/xAb VH CDR2 (Contact)
WMGWINTYTGEPT

SEQ ID NO: 10 - protein, 8 aa, Artificial Sequence
  Antibody z10/z11/z13/xAb VH CDR2 (IMGT)
INTYTGEP

SEQ ID NO: 11 - protein, 11 aa, Artificial Sequence
  Antibody z10/z11/z13/xAb VH CDR3 (Kabat/AbM/Exemplary)
KSTVVSRYFDV

SEQ ID NO: 12 - protein, 9 aa, Artificial Sequence
  Antibody z10/z11/z13/xAb VH CDR3 (Chothia)
STVVSRYFD

SEQ ID NO: 13 - protein, 12 aa, Artificial Sequence
  Antibody z10/z11/z13/xAb VH CDR3 (Contact)
ARKSTVVSRYFD

SEQ ID NO: 14 - protein, 13 aa, Artificial Sequence
  Antibody z10/z11/z13/xAb VH CDR3 (IMGT)
ARKSTVVSRYFDV

SEQ ID NO: 15 - protein, 30 aa, Artificial Sequence
  Antibody z10/Z11/z13 VH Framework Region VH FR1 (Kabat)
QVQLVQSGAEVKKPGASVKVSCKASGYTFT

SEQ ID NO: 16 - protein, 14 aa, Artificial Sequence
  Antibody z10/z11/z13 VH Framework Region VH FR2 (Kabat)
WVRQAPGQGLEWMG

SEQ ID NO: 17 - protein, 32 aa, Artificial Sequence
  Antibody z10 VH Framework Region VH FR3 (Kabat/Exemplary)
RVTFTTDTSTSTAYMELRSLRSDDMAVYYCAR

SEQ ID NO: 18 - protein, 11 aa, Artificial Sequence
  Antibody z10/z11/z13 VH Framework Region VH FR4 (Kabat)
WGQGTTVTVSS

SEQ ID NO: 19 - protein, 25 aa, Artificial Sequence [sequence omitted]

SEQ ID NO: 20 - protein, 20 aa, Artificial Sequence
  Antibody z10/z11/z13 VH Framework Region VH FR2 (Chothia)
GMNWVRQAPGQGLEWMGWIN

SEQ ID NO: 21 - protein, 43 aa, Artificial Sequence
  Antibody z10 VH Framework Region VH FR3 (Chothia)
EPTYADDFKGRVTFTTDTSTSTAYMELRSLRSDDMAVYYCARK

SEQ ID NO: 22 - protein, 12 aa, Artificial Sequence
  Antibody z10/z11/z13 VH Framework Region VH FR4 (Chothia)
VWGQGTTVTVSS

SEQ ID NO: 23 - protein, 25 aa, Artificial Sequence [sequence omitted]

SEQ ID NO: 24 - protein, 14 aa, Artificial Sequence
  Antibody z10/z11/z13 VH Framework Region VH FR2 (AbM)
WVRQAPGQGLEWMG

SEQ ID NO: 25 - protein, 39 aa, Artificial Sequence
  Antibody z10 VH Framework Region VH FR3 (AbM)
YADDFKGRVTFTTDTSTSTAYMELRSLRSDDMAVYYCAR

SEQ ID NO: 26 - protein, 11 aa, Artificial Sequence
  Antibody z10/z11/z13 VH Framework Region VH FR4 (AbM)
WGQGTTVTVSS

SEQ ID NO: 27 - protein, 29 aa, Artificial Sequence
  Antibody z10/z11/z13 VH Framework Region VH FR1 (Contact)
QVQLVQSGAEVKKPGASVKVSCKASGYTF

SEQ ID NO: 28 - protein, 11 aa, Artificial Sequence
  Antibody z10/z11/z13 VH Framework Region VH FR2 (Contact)
WVRQAPGQGLE

SEQ ID NO: 29 - protein, 37 aa, Artificial Sequence
  Antibody z10 VH Framework Region VH FR3 (Contact)
YADDFKGRVTFTTDTSTSTAYMELRSLRSDDMAVYYC

SEQ ID NO: 30 - protein, 12 aa, Artificial Sequence
  Antibody z10/z11/z13 VH Framework Region VH FR4 (Contact)
VWGQGTTVTVSS

SEQ ID NO: 31 - protein, 25 aa, Artificial Sequence [sequence omitted]

SEQ ID NO: 32 - protein, 17 aa, Artificial Sequence
  Antibody z10/z11/z13 VH Framework Region VH FR2 (IMGT)
MNWVRQAPGQGLEWMGW

SEQ ID NO: 33 - protein, 38 aa, Artificial Sequence
  Antibody z10 VH Framework Region VH FR3 (IMGT)
TYADDFKGRVTFTTDTSTSTAYMELRSLRSDDMAVYYC

SEQ ID NO: 34 - protein, 11 aa, Artificial Sequence
  Antibody z10/z11/z13 VH Framework Region VH FR4 (IMGT)
WGQGTTVTVSS

SEQ ID NO: 35 - protein, 25 aa, Artificial Sequence [sequence omitted]

SEQ ID NO: 36 - protein, 14 aa, Artificial Sequence
  Antibody z10/z11/z13 VH Framework Region VH FR2 (Exemplary)
WVRQAPGQGLEWMG

SEQ ID NO: 37 - protein, 11 aa, Artificial Sequence
  Antibody z10/z11/z13 VH Framework Region VH FR4 (Exemplary)
WGQGTTVTVSS

SEQ ID NO: 38 - protein, 32 aa, Artificial Sequence
  Antibody z11 VH Framework Region VH FR3 (Kabat/Exemplary)
RVTMTLDTSTSTAYMELRSLRSDDMAVYYCAR

SEQ ID NO: 39 - protein, 43 aa, Artificial Sequence
  Antibody z11 VH Framework Region VH FR3 (Chothia)
EPTYADDFKGRVTMTLDTSTSTAYMELRSLRSDDMAVYYCARK

SEQ ID NO: 40 - protein, 39 aa, Artificial Sequence
  Antibody z11 VH Framework Region VH FR3 (AbM)
YADDFKGRVTMTLDTSTSTAYMELRSLRSDDMAVYYCAR

SEQ ID NO: 41 - protein, 37 aa, Artificial Sequence
  Antibody z11 VH Framework Region VH FR3 (Contact)
YADDFKGRVTMTLDTSTSTAYMELRSLRSDDMAVYYC

SEQ ID NO: 42 - protein, 38 aa, Artificial Sequence
  Antibody z11 VH Framework Region VH FR3 (IMGT)
TYADDFKGRVTMTLDTSTSTAYMELRSLRSDDMAVYYC

SEQ ID NO: 43 - protein, 32 aa, Artificial Sequence
  Antibody z13 VH Framework Region VH FR3 (Kabat/Exemplary)
RVTFTLDTSTSTAYMELRSLRSDDMAVYYCAR

SEQ ID NO: 44 - protein, 43 aa, Artificial Sequence
  Antibody z13 VH Framework Region VH FR3 (Chothia)
EPTYADDFKGRVTFTLDTSTSTAYMELRSLRSDDMAVYYCARK

SEQ ID NO: 45 - protein, 39 aa, Artificial Sequence
  Antibody z13 VH Framework Region VH FR3 (AbM)
YADDFKGRVTFTLDTSTSTAYMELRSLRSDDMAVYYCAR

SEQ ID NO: 46 - protein, 37 aa, Artificial Sequence
  Antibody z13 VH Framework Region VH FR3 (Contact)
YADDFKGRVTFTLDTSTSTAYMELRSLRSDDMAVYYC

SEQ ID NO: 47 - protein, 38 aa, Artificial Sequence
  Antibody z13 VH Framework Region VH FR3 (IMGT)
TYADDFKGRVTFTLDTSTSTAYMELRSLRSDDMAVYYC

SEQ ID NO: 48 - protein, 32 aa, Artificial Sequence
  Antibody VH FR3 Consensus sequence (Kabat)
  misc_feature (4)..(4): Xaa = Phe or Met
  misc_feature (6)..(6): Xaa = Thr or Leu
RVTXTXDTSTSTAYMELRSLRSDDMAVYYCAR

SEQ ID NO: 49 - protein, 43 aa, Artificial Sequence
  Antibody VH FR3 Consensus sequence (Chothia)
  misc_feature (14)..(14): Xaa = Phe or Met
  misc_feature (16)..(16): Xaa = Thr or Leu
EPTYADDFKGRVTXTXDTSTSTAYMELRSLRSDDMAVYYCARK

SEQ ID NO: 50 - protein, 39 aa, Artificial Sequence
  Antibody VH FR3 Consensus sequence (AbM)
  misc_feature (11)..(11): Xaa = Phe or Met
  misc_feature (13)..(13): Xaa = Thr or Leu
YADDFKGRVTXTXDTSTSTAYMELRSLRSDDMAVYYCAR

SEQ ID NO: 51 - protein, 37 aa, Artificial Sequence
  Antibody VH FR3 Consensus sequence (Contact)
  misc_feature (11)..(11): Xaa = Phe or Met
  misc_feature (13)..(13): Xaa = Thr or Leu
YADDFKGRVTXTXDTSTSTAYMELRSLRSDDMAVYYC

SEQ ID NO: 52 - protein, 38 aa, Artificial Sequence
  Antibody VH FR3 Consensus sequence (IMGT)
  misc_feature (12)..(12): Xaa = Phe or Met
  misc_feature (14)..(14): Xaa = Thr or Leu
TYADDFKGRVTXTXDTSTSTAYMELRSLRSDDMAVYYC

SEQ ID NO: 53 - protein, 32 aa, Artificial Sequence; identical to SEQ ID NO: 48
  Antibody VH FR3 Consensus sequence (Exemplary)
  misc_feature (4)..(4): Xaa = Phe or Met
  misc_feature (6)..(6): Xaa = Thr or Leu

SEQ ID NO: 54 - protein, 30 aa, Artificial Sequence
  Antibody xAb VH Framework Region VH FR1 (Kabat)
QIQLVQSGPELKKPGETVKISCKASGYTFT

SEQ ID NO: 55 - protein, 14 aa, Artificial Sequence
  Antibody xAb VH Framework Region VH FR2 (Kabat/AbM/Exemplary)
WVKQAPGKGLKWMG

SEQ ID NO: 56 - protein, 32 aa, Artificial Sequence
  Antibody xAb VH Framework Region VH FR3 (Kabat/Exemplary)
RFVFSLETSASTAYLQINNLKNEDMATYFCAR

SEQ ID NO: 57 - protein, 11 aa, Artificial Sequence
  Antibody xAb VH Framework Region VH FR4 (Kabat/AbM/IMGT/Exemplary)
WGAGTTVTVSS

SEQ ID NO: 58 - protein, 25 aa, Artificial Sequence
  Antibody xAb VH Framework Region VH FR1 (Chothia/AbM/IMGT/Exemplary)
QIQLVQSGPELKKPGETVKISCKAS

SEQ ID NO: 59 - protein, 20 aa, Artificial Sequence
  Antibody xAb VH Framework Region VH FR2 (Chothia)
GMNWVKQAPGKGLKWMGWIN

SEQ ID NO: 60 - protein, 43 aa, Artificial Sequence
  Antibody xAb VH Framework Region VH FR3 (Chothia)
EPTYADDFKGRFVFSLETSASTAYLQINNLKNEDMATYFCARK

SEQ ID NO: 61 - protein, 12 aa, Artificial Sequence
  Antibody xAb VH Framework Region VH FR4 (Chothia/Contact)
VWGAGTTVTVSS

SEQ ID NO: 62 - protein, 39 aa, Artificial Sequence
  Antibody xAb VH Framework Region VH FR3 (AbM)
YADDFKGRFVFSLETSASTAYLQINNLKNEDMATYFCAR

SEQ ID NO: 63 - protein, 29 aa, Artificial Sequence
  Antibody xAb VH Framework Region VH FR1 (Contact)
QIQLVQSGPELKKPGETVKISCKASGYTF

SEQ ID NO: 64 - protein, 11 aa, Artificial Sequence
  Antibody xAb VH Framework Region VH FR2 (Contact)
WVKQAPGKGLK

SEQ ID NO: 65 - protein, 37 aa, Artificial Sequence
  Antibody xAb VH Framework Region VH FR3 (Contact)
YADDFKGRFVFSLETSASTAYLQINNLKNEDMATYFC

SEQ ID NO: 66 - protein, 17 aa, Artificial Sequence
  Antibody xAb VH Framework Region VH FR2 (IMGT)
MNWVKQAPGKGLKWMGW

SEQ ID NO: 67 - protein, 38 aa, Artificial Sequence
  Antibody xAb VH Framework Region VH FR3 (IMGT)
TYADDFKGRFVFSLETSASTAYLQINNLKNEDMATYFC

SEQ ID NO: 68 - protein, 11 aa, Artificial Sequence
  Antibody z10/z11/z13/xAb VL CDR1 (Kabat/AbM/Exemplary)
KASQDVGDAVT

SEQ ID NO: 69 - protein, 7 aa, Artificial Sequence
  Antibody z10/z11/z13/xAb VL CDR2 (Kabat/AbM/Exemplary)
WASTRHT

SEQ ID NO: 70 - protein, 9 aa, Artificial Sequence
  Antibody z10/z11/z13/xAb VL CDR3 (Kabat/AbM/IMGT/Exemplary)
QQYRSYPLT

SEQ ID NO: 71 - protein, 7 aa, Artificial Sequence
  Antibody z10/z11/z13/xAb VL CDR1 (Chothia)
SQDVGDA

SEQ ID NO: 72 - protein, 3 aa, Artificial Sequence
  Antibody z10/z11/z13/xAb VL CDR2 (Chothia/IMGT)
WAS

SEQ ID NO: 73 - protein, 6 aa, Artificial Sequence
  Antibody z10/z11/z13/xAb VL CDR3 (Chothia)
YRSYPL

SEQ ID NO: 74 - protein, 7 aa, Artificial Sequence
  Antibody z10/z11/z13 VL CDR1 (Contact)
GDAVTWY

SEQ ID NO: 75 - protein, 10 aa, Artificial Sequence
  Antibody z10/z11/z13/xAb VL CDR2 (Contact)
LLIYWASTRH

SEQ ID NO: 76 - protein, 8 aa, Artificial Sequence
  Antibody z10/z11/z13/xAb VL CDR3 (Contact)
QQYRSYPL

SEQ ID NO: 77 - protein, 6 aa, Artificial Sequence
  Antibody z10/z11/z13/xAb VL CDR1 (IMGT)
QDVGDA

SEQ ID NO: 78 - protein, 7 aa, Artificial Sequence
  Antibody xAb VL CDR1 (Contact)
GDAVTWC

SEQ ID NO: 79 - protein, 23 aa, Artificial Sequence
  Antibody z10/z11/z13 VL Framework Region VL FR1 (Kabat/AbM/Exemplary)
DIQMTQSPSFLSASVGDRVTITC

SEQ ID NO: 80 - protein, 15 aa, Artificial Sequence
  Antibody z10/z11/z13 VL Framework Region VL FR2 (Kabat/AbM/Exemplary)
WYQQKPGKAPKLLIY

SEQ ID NO: 81 - protein, 32 aa, Artificial Sequence
  Antibody z10/z11/z13 VL Framework Region VL FR3 (Kabat/AbM/Exemplary)
GVPDRFSGSGSGTDFTLTISSLQPEDFATYYC

SEQ ID NO: 82 - protein, 10 aa, Artificial Sequence
  Antibody z10/z11/z13 VL Framework Region VL FR4 (Kabat/AbM/IMGT/Exemplary)
FGQGTKLEIK

SEQ ID NO: 83 - protein, 25 aa, Artificial Sequence
  Antibody z10/z11/z13 VL Framework Region VL FR1 (Chothia)
DIQMTQSPSFLSASVGDRVTITCKA

SEQ ID NO: 84 - protein, 17 aa, Artificial Sequence
  Antibody z10/z11/z13 VL Framework Region VL FR2 (Chothia/IMGT)
VTWYQQKPGKAPKLLIY

SEQ ID NO: 85 - protein, 38 aa, Artificial Sequence
  Antibody z10/z11/z13 VL Framework Region VL FR3 (Chothia)
TRHTGVPDRFSGSGSGTDFTLTISSLQPEDFATYYCQQ

SEQ ID NO: 86 - protein, 11 aa, Artificial Sequence
  Antibody z10/z11/z13 VL Framework Region VL FR4 (Chothia/Contact)
TFGQGTKLEIK

SEQ ID NO: 87 - protein, 29 aa, Artificial Sequence
  Antibody z10/z11/z13 VL Framework Region VL FR1 (Contact)
DIQMTQSPSFLSASVGDRVTITCKASQDV

SEQ ID NO: 88 - protein, 9 aa, Artificial Sequence
  Antibody z10/z11/z13 VL Framework Region VL FR2 (Contact)
QQKPGKAPK

SEQ ID NO: 89 - protein, 33 aa, Artificial Sequence
  Antibody z10/z11/z13 VL Framework Region VL FR3 (Contact)
TGVPDRFSGSGSGTDFTLTISSLQPEDFATYYC

SEQ ID NO: 90 - protein, 26 aa, Artificial Sequence
  Antibody z10/z11/z13 VL Framework Region VL FR1 (IMGT)
DIQMTQSPSFLSASVGDRVTITCKAS

SEQ ID NO: 91 - protein, 36 aa, Artificial Sequence
  Antibody z10/z11/z13 VL Framework Region VL FR3 (IMGT)
TRHTGVPDRFSGSGSGTDFTLTISSLQPEDFATYYC

SEQ ID NO: 92 - protein, 23 aa, Artificial Sequence
  Antibody xAb VL Framework Region VL FR1 (Kabat/AbM/Exemplary)
DIVLTQSHKFMSTSVGDRVSITC

SEQ ID NO: 93 - protein, 15 aa, Artificial Sequence
  Antibody xAb VL Framework Region VL FR2 (Kabat/AbM/Exemplary)
WCQQKPGQPPKLLIY

SEQ ID NO: 94 - protein, 32 aa, Artificial Sequence
  Antibody xAb VL Framework Region VL FR3 (Kabat/AbM/Exemplary)
GVPDRFTGSGSGTDFTLTINNVQSEDLADYFC

SEQ ID NO: 95 - protein, 10 aa, Artificial Sequence
  Antibody xAb VL Framework Region VL FR4 (Kabat/AbM/IMGT/Exemplary)
FGAGTKLELK

SEQ ID NO: 96 - protein, 25 aa, Artificial Sequence
  Antibody xAb VL Framework Region VL FR1 (Chothia)
DIVLTQSHKFMSTSVGDRVSITCKA

SEQ ID NO: 97 - protein, 17 aa, Artificial Sequence
  Antibody xAb VL Framework Region VL FR2 (Chothia/IMGT)
VTWCQQKPGQPPKLLIY

SEQ ID NO: 98 - protein, 38 aa, Artificial Sequence
  Antibody xAb VL Framework Region VL FR3 (Chothia)
TRHTGVPDRFTGSGSGTDFTLTINNVQSEDLADYFCQQ

SEQ ID NO: 99 - protein, 11 aa, Artificial Sequence
  Antibody xAb VL Framework Region VL FR4 (Chothia/Contact)
TFGAGTKLELK

SEQ ID NO: 100 - protein, 29 aa, Artificial Sequence
  Antibody xAb VL Framework Region VL FR1 (Contact)
DIVLTQSHKFMSTSVGDRVSITCKASQDV

SEQ ID NO: 101 - protein, 9 aa, Artificial Sequence
  Antibody xAb VL Framework Region VL FR2 (Contact)
QQKPGQPPK

SEQ ID NO: 102 - protein, 33 aa, Artificial Sequence
  Antibody xAb VL Framework Region VL FR3 (Contact)
TGVPDRFTGSGSGTDFTLTINNVQSEDLADYFC

SEQ ID NO: 103 - protein, 26 aa, Artificial Sequence
  Antibody xAb VL Framework Region VL FR1 (IMGT)
DIVLTQSHKFMSTSVGDRVSITCKAS

SEQ ID NO: 104 - protein, 36 aa, Artificial Sequence
  Antibody xAb VL Framework Region VL FR3 (IMGT)
TRHTGVPDRFTGSGSGTDFTLTINNVQSEDLADYFC

SEQ ID NO: 105 - protein, 120 aa, Artificial Sequence
  Antibody z10 Heavy Chain Variable Region (VH)
QVQLVQSGAEVKKPGASVKVSCKASGYTFTNYGMNWVRQAPGQGLEWMGWINTYTGEPTYADDFKGRVTFTTDTSTSTAYMELRSLRSDDMAVYYCARKSTVVSRYFDVWGQGTTVTVSS

SEQ ID NO: 106 - protein, 107 aa, Artificial Sequence
  Antibody z10/z11/z13 light Chain Variable Region (VL)
DIQMTQSPSFLSASVGDRVTITCKASQDVGDAVTWYQQKPGKAPKLLIYWASTRHTGVPDRFSGSGSGTDFTLTISSLQPEDFATYYCQQYRSYPLTFGQGTKLEIK

SEQ ID NO: 107 - protein, 120 aa, Artificial Sequence
  Antibody z11 Heavy Chain Variable Region (VH)
QVQLVQSGAEVKKPGASVKVSCKASGYTFTNYGMNWVRQAPGQGLEWMGWINTYTGEPTYADDFKGRVTMTLDTSTSTAYMELRSLRSDDMAVYYCARKSTVVSRYFDVWGQGTTVTVSS

SEQ ID NO: 108 - protein, 120 aa, Artificial Sequence
  Antibody z13 Heavy Chain Variable Region (VH)
QVQLVQSGAEVKKPGASVKVSCKASGYTFTNYGMNWVRQAPGQGLEWMGWINTYTGEPTYADDFKGRVTFTLDTSTSTAYMELRSLRSDDMAVYYCARKSTVVSRYFDVWGQGTTVTVSS

SEQ ID NO: 109 - protein, 120 aa, Artificial Sequence
  Antibody Heavy Chain Variable Region Consensus sequence
  misc_feature (70)..(70): Xaa = Phe or Met
  misc_feature (72)..(72): Xaa =  Thr or Leu
QVQLVQSGAEVKKPGASVKVSCKASGYTFTNYGMNWVRQAPGQGLEWMGWINTYTGEPTYADDFKGRVTXTXDTSTSTAYMELRSLRSDDMAVYYCARKSTVVSRYFDVWGQGTTVTVSS

SEQ ID NO: 110 - protein, 120 aa, Artificial Sequence
  Antibody xAb Heavy Chain Variable Region (VH)
QIQLVQSGPELKKPGETVKISCKASGYTFTNYGMNWVKQAPGKGLKWMGWINTYTGEPTYADDFKGRFVFSLETSASTAYLQINNLKNEDMATYFCARKSTVVSRYFDVWGAGTTVTVSS

SEQ ID NO: 111 - protein, 107 aa, Artificial Sequence
  Antibody xAb Light Chain Variable Region (VL)
DIVLTQSHKFMSTSVGDRVSITCKASQDVGDAVTWCQQKPGQPPKLLIYWASTRHTGVPDRFTGSGSGTDFTLTINNVQSEDLADYFCQQYRSYPLTFGAGTKLELK

SEQ ID NO: 112 - protein, 450 aa, Artificial Sequence
  Antibody z10 Heavy Chain
QVQLVQSGAEVKKPGASVKVSCKASGYTFTNYGMNWVRQAPGQGLEWMGWINTYTGEPTYADDFKGRVTFTTDTSTSTAYMELRSLRSDDMAVYYCARKSTVVSRYFDVWGQGTTVTVSSASTKGPSVFPLAPSSKSTSGGTAALGCLVKDYFPEPVTVSWNSGALTSGVHTFPAVLQSSGLYSLSSVVTVPSSSLGTQTYICNVNHKPSNTKVDKRVEPKSCDKTHTCPPCPAPELLGGPSVFLFPPKPKDTLMISRTPEVTCVVVDVSHEDPEVKFNWYVDGVEVHNAKTKPREEQYNSTYRVVSVLTVLHQDWLNGKEYKCKVSNKALPAPIEKTISKAKGQPREPQVYTLPPSREEMTKNQVSLTCLVKGFYPSDIAVEWESNGQPENNYKTTPPVLDSDGSFFLYSKLTVDKSRWQQGNVFSCSVMHEALHNHYTQKSLSLSPGK

SEQ ID NO: 113 - protein, 214 aa, Artificial Sequence
  Antibody z10/z11/z13 Light Chain
DIQMTQSPSFLSASVGDRVTITCKASQDVGDAVTWYQQKPGKAPKLLIYWASTRHTGVPDRFSGSGSGTDFTLTISSLQPEDFATYYCQQYRSYPLTFGQGTKLEIKRTVAAPSVFIFPPSDEQLKSGTASVVCLLNNFYPREAKVQWKVDNALQSGNSQESVTEQDSKDSTYSLSSTLTLSKADYEKHKVYACEVTHQGLSSPVTKSFNRGEC

SEQ ID NO: 114 - protein, 450 aa, Artificial Sequence
  Antibody z11 Heavy Chain
QVQLVQSGAEVKKPGASVKVSCKASGYTFTNYGMNWVRQAPGQGLEWMGWINTYTGEPTYADDFKGRVTMTLDTSTSTAYMELRSLRSDDMAVYYCARKSTVVSRYFDVWGQGTTVTVSSASTKGPSVFPLAPSSKSTSGGTAALGCLVKDYFPEPVTVSWNSGALTSGVHTFPAVLQSSGLYSLSSVVTVPSSSLGTQTYICNVNHKPSNTKVDKRVEPKSCDKTHTCPPCPAPELLGGPSVFLFPPKPKDTLMISRTPEVTCVVVDVSHEDPEVKFNWYVDGVEVHNAKTKPREEQYNSTYRVVSVLTVLHQDWLNGKEYKCKVSNKALPAPIEKTISKAKGQPREPQVYTLPPSREEMTKNQVSLTCLVKGFYPSDIAVEWESNGQPENNYKTTPPVLDSDGSFFLYSKLTVDKSRWQQGNVFSCSVMHEALHNHYTQKSLSLSPGK

SEQ ID NO: 115 - protein, 450 aa, Artificial Sequence
  Antibody z13 Heavy Chain
QVQLVQSGAEVKKPGASVKVSCKASGYTFTNYGMNWVRQAPGQGLEWMGWINTYTGEPTYADDFKGRVTFTLDTSTSTAYMELRSLRSDDMAVYYCARKSTVVSRYFDVWGQGTTVTVSSASTKGPSVFPLAPSSKSTSGGTAALGCLVKDYFPEPVTVSWNSGALTSGVHTFPAVLQSSGLYSLSSVVTVPSSSLGTQTYICNVNHKPSNTKVDKRVEPKSCDKTHTCPPCPAPELLGGPSVFLFPPKPKDTLMISRTPEVTCVVVDVSHEDPEVKFNWYVDGVEVHNAKTKPREEQYNSTYRVVSVLTVLHQDWLNGKEYKCKVSNKALPAPIEKTISKAKGQPREPQVYTLPPSREEMTKNQVSLTCLVKGFYPSDIAVEWESNGQPENNYKTTPPVLDSDGSFFLYSKLTVDKSRWQQGNVFSCSVMHEALHNHYTQKSLSLSPGK

SEQ ID NO: 116 - protein, 450 aa, Artificial Sequence
  Antibody Heavy Chain Consensus Sequences
  misc_feature (70)..(70): Xaa = Phe or Met
  misc_feature (72)..(72): Xaa = Thr or Leu
QVQLVQSGAEVKKPGASVKVSCKASGYTFTNYGMNWVRQAPGQGLEWMGWINTYTGEPTYADDFKGRVTXTXDTSTSTAYMELRSLRSDDMAVYYCARKSTVVSRYFDVWGQGTTVTVSSASTKGPSVFPLAPSSKSTSGGTAALGCLVKDYFPEPVTVSWNSGALTSGVHTFPAVLQSSGLYSLSSVVTVPSSSLGTQTYICNVNHKPSNTKVDKRVEPKSCDKTHTCPPCPAPELLGGPSVFLFPPKPKDTLMISRTPEVTCVVVDVSHEDPEVKFNWYVDGVEVHNAKTKPREEQYNSTYRVVSVLTVLHQDWLNGKEYKCKVSNKALPAPIEKTISKAKGQPREPQVYTLPPSREEMTKNQVSLTCLVKGFYPSDIAVEWESNGQPENNYKTTPPVLDSDGSFFLYSKLTVDKSRWQQGNVFSCSVMHEALHNHYTQKSLSLSPGK

SEQ ID NO: 117 - protein, 450 aa, Artificial Sequence
  Antibody xAb Heavy Chain
QIQLVQSGPELKKPGETVKISCKASGYTFTNYGMNWVKQAPGKGLKWMGWINTYTGEPTYADDFKGRFVFSLETSASTAYLQINNLKNEDMATYFCARKSTVVSRYFDVWGAGTTVTVSSASTKGPSVFPLAPSSKSTSGGTAALGCLVKDYFPEPVTVSWNSGALTSGVHTFPAVLQSSGLYSLSSVVTVPSSSLGTQTYICNVNHKPSNTKVDKRVEPKSCDKTHTCPPCPAPELLGGPSVFLFPPKPKDTLMISRTPEVTCVVVDVSHEDPEVKFNWYVDGVEVHNAKTKPREEQYNSTYRVVSVLTVLHQDWLNGKEYKCKVSNKALPAPIEKTISKAKGQPREPQVYTLPPSREEMTKNQVSLTCLVKGFYPSDIAVEWESNGQPENNYKTTPPVLDSDGSFFLYSKLTVDKSRWQQGNVFSCSVMHEALHNHYTQKSLSLSPGK

SEQ ID NO: 118 - protein, 214 aa, Artificial Sequence
  Antibody xAb Light Chain
DIVLTQSHKFMSTSVGDRVSITCKASQDVGDAVTWCQQKPGQPPKLLIYWASTRHTGVPDRFTGSGSGTDFTLTINNVQSEDLADYFCQQYRSYPLTFGAGTKLELKRTVAAPSVFIFPPSDEQLKSGTASVVCLLNNFYPREAKVQWKVDNALQSGNSQESVTEQDSKDSTYSLSSTLTLSKADYEKHKVYACEVTHQGLSSPVTKSFNRGEC

SEQ ID NO: 119 - DNA, 360 bp, Artificial Sequence
  Antibody z10 Variable Region VH DNA Sequences
caggtgcagctggtgcagagcggcgctgaggtgaagaagcccggcgctagcgtgaaggtgagctgcaaggccagcggctacaccttcaccaactacggcatgaactgggtgaggcaggctcctggacagggcctggagtggatgggctggatcaacacatacaccggcgagcccacctacgccgacgacttcaagggcagggtgacctttaccaccgacaccagcaccagcaccgcctacatggagctgaggagcctgagaagcgacgacatggccgtgtactactgcgccagaaagagcaccgtggtgtccaggtacttcgacgtgtggggccagggcaccacagtgaccgtgagcagc

SEQ ID NO: 120 - DNA, 321 bp, Artificial Sequence
  Antibody z10/z11/z13 Variable Region VL DNA Sequences
gacatccagatgacccagagccccagcttcctgtccgctagcgtgggcgacagggtgaccatcacctgcaaggccagccaggacgtgggcgatgccgtgacctggtatcagcagaagcccggcaaggcccccaagctgctgatctactgggccagcacaaggcacacaggcgtgcccgacagattcagcggcagcggaagcggcaccgacttcaccctgaccatcagcagcctgcagcccgaggacttcgccacctactactgccagcagtacaggagctaccccctgaccttcggccagggcaccaagctggaaatcaag

SEQ ID NO: 121 - DNA, 360 bp, Artificial Sequence
  Antibody z11 Variable Region VH DNA Sequences
caggtgcagctggtgcagagcggagccgaggtgaagaagcctggcgccagcgtgaaggtgagctgcaaggccagcggctacaccttcaccaactacggcatgaactgggtgaggcaggctcctggccagggactggagtggatgggctggatcaacacctacaccggcgagcccacctacgccgacgacttcaagggcagggtgaccatgaccctggacaccagcaccagcaccgcctacatggagctgaggagcctgaggagcgacgacatggccgtgtactactgcgccaggaagagcaccgtggtgtccaggtacttcgacgtgtggggacagggcaccaccgtgaccgtgagcagc

SEQ ID NO: 122 - DNA, 360 bp, Artificial Sequence
  Antibody z13 Variable Region VH DNA Sequences
caggtgcagctggtgcagagcggagccgaagtgaagaagcccggcgccagcgtgaaggtgagctgcaaggccagcggctacaccttcaccaactacggcatgaactgggtgagacaggcccctggacagggactggagtggatgggctggatcaacacctacaccggcgagcccacctacgccgacgacttcaagggcagggtgaccttcaccctggacaccagcaccagcaccgcctacatggagctgaggagcctgaggagcgacgacatggccgtgtactattgcgccaggaagagcaccgtggtgagcaggtacttcgacgtgtggggccagggaaccaccgtgaccgtgagcagc

SEQ ID NO: 123 - DNA, 360 bp, Artificial Sequence
  Antibody xAb Variable Region VH DNA Sequences
cagatccagttggtgcagtctggacctgagctgaagaagcctggagagacagtcaagatctcctgcaaggcttctggatataccttcacaaactatggaatgaactgggtgaagcaggctccaggaaagggtttaaagtggatgggctggataaacacctacactggagagccaacatatgctgatgacttcaagggacggtttgtcttctctttggaaacctctgccagcactgcctacttgcagatcaacaacctcaaaaatgaggacatggccacatatttctgtgcaagaaaaagtacggtagtaagtaggtacttcgatgtctggggcgcagggaccacggtcaccgtctcctca

SEQ ID NO: 124 - DNA, 321 bp, Artificial Sequence
  Antibody xAb Variable Region VL DNA Sequences
gacattgtgctgacccagtctcacaaattcatgtccacatcagtaggagacagggtcagcatcacctgcaaggccagtcaggatgtgggtgatgctgtaacctggtgtcaacagaaaccaggtcaacctcctaaactactgatttactgggcatccacccggcacactggagtccctgatcgcttcacaggcagtgggtctgggacagatttcactctcaccattaacaatgtgcagtctgaggacttggcagattatttctgtcagcaatatcgcagctatcctctcacgttcggtgctgggaccaagctggagctgaaa

SEQ ID NO: 125 - DNA, 1353 bp, Artificial Sequence
  Antibody z10 Heavy Chain DNA Sequences
caggtgcagctggtgcagagcggcgctgaggtgaagaagcccggcgctagcgtgaaggtgagctgcaaggccagcggctacaccttcaccaactacggcatgaactgggtgaggcaggctcctggacagggcctggagtggatgggctggatcaacacatacaccggcgagcccacctacgccgacgacttcaagggcagggtgacctttaccaccgacaccagcaccagcaccgcctacatggagctgaggagcctgagaagcgacgacatggccgtgtactactgcgccagaaagagcaccgtggtgtccaggtacttcgacgtgtggggccagggcaccacagtgaccgtgagcagcgcgtcgaccaagggcccatccgtcttccccctggcaccctcctccaagagcacctctgggggcacagcggccctgggctgcctggtcaaggactacttccccgaaccggtgacggtgtcctggaactcaggcgctctgaccagcggcgtgcacaccttcccggctgtcctacagtcctcaggactctactccctcagcagcgtggtgaccgtgccctccagcagcttgggcacccagacctacatctgcaacgtgaatcacaagcccagcaacaccaaggtggacaagagagttgagcccaaatcttgtgacaaaactcacacatgcccaccgtgcccagcacctgaactcctggggggaccgtcagtcttcctcttccccccaaaacccaaggacaccctcatgatctcccggacccctgaggtcacatgcgtggtggtggacgtgagccacgaagaccctgaggtcaagttcaactggtacgtggacggcgtggaggtgcataatgccaagacaaagccgcgggaggagcagtacaacagcacgtaccgtgtggtcagcgtcctcaccgtcctgcaccaggactggctgaatggcaaggagtacaagtgcaaggtctccaacaaagccctcccagcccccatcgagaaaaccatctccaaagccaaagggcagccccgagaaccacaggtctacaccctgcccccatcccgggaggagatgaccaagaaccaggtcagcctgacctgcctggtcaaaggcttctatcccagcgacatcgccgtggagtgggagagcaatgggcagccggagaacaactacaagaccacgcctcccgtgctggactccgacggctccttcttcctctatagcaagctcaccgtggacaagagcaggtggcagcaggggaacgtcttctcatgctccgtgatgcatgaggctctgcacaaccactacacgcagaagagcttaagcctgtctccgggtaaatga

SEQ ID NO: 126 - DNA, 645 bp, Artificial Sequence
  Antibody z10/z11/z13 Light Chain DNA Sequences
gacatccagatgacccagagccccagcttcctgtccgctagcgtgggcgacagggtgaccatcacctgcaaggccagccaggacgtgggcgatgccgtgacctggtatcagcagaagcccggcaaggcccccaagctgctgatctactgggccagcacaaggcacacaggcgtgcccgacagattcagcggcagcggaagcggcaccgacttcaccctgaccatcagcagcctgcagcccgaggacttcgccacctactactgccagcagtacaggagctaccccctgaccttcggccagggcaccaagctggaaatcaagcgtacggtggctgcaccatctgtcttcatcttcccgccatctgatgagcagttgaaatctggaactgcctctgttgtgtgcctgctgaataacttctatcccagagaggccaaagtacagtggaaggtggataacgccctccaatcgggtaactcccaggagagtgtcacagagcaggacagcaaggacagcacctacagcctcagcagcaccctgacgctgagcaaagcagactacgagaaacacaaagtctacgcctgcgaagtcacccatcagggcctgagctcgcccgtcacaaagagcttcaacaggggagagtgttga

SEQ ID NO: 127 - DNA, 1353 bp, Artificial Sequence
  Antibody z11 Heavy Chain DNA Sequences
caggtgcagctggtgcagagcggagccgaggtgaagaagcctggcgccagcgtgaaggtgagctgcaaggccagcggctacaccttcaccaactacggcatgaactgggtgaggcaggctcctggccagggactggagtggatgggctggatcaacacctacaccggcgagcccacctacgccgacgacttcaagggcagggtgaccatgaccctggacaccagcaccagcaccgcctacatggagctgaggagcctgaggagcgacgacatggccgtgtactactgcgccaggaagagcaccgtggtgtccaggtacttcgacgtgtggggacagggcaccaccgtgaccgtgagcagcgcgtcgaccaagggcccatccgtcttccccctggcaccctcctccaagagcacctctgggggcacagcggccctgggctgcctggtcaaggactacttccccgaaccggtgacggtgtcctggaactcaggcgctctgaccagcggcgtgcacaccttcccggctgtcctacagtcctcaggactctactccctcagcagcgtggtgaccgtgccctccagcagcttgggcacccagacctacatctgcaacgtgaatcacaagcccagcaacaccaaggtggacaagagagttgagcccaaatcttgtgacaaaactcacacatgcccaccgtgcccagcacctgaactcctggggggaccgtcagtcttcctcttccccccaaaacccaaggacaccctcatgatctcccggacccctgaggtcacatgcgtggtggtggacgtgagccacgaagaccctgaggtcaagttcaactggtacgtggacggcgtggaggtgcataatgccaagacaaagccgcgggaggagcagtacaacagcacgtaccgtgtggtcagcgtcctcaccgtcctgcaccaggactggctgaatggcaaggagtacaagtgcaaggtctccaacaaagccctcccagcccccatcgagaaaaccatctccaaagccaaagggcagccccgagaaccacaggtctacaccctgcccccatcccgggaggagatgaccaagaaccaggtcagcctgacctgcctggtcaaaggcttctatcccagcgacatcgccgtggagtgggagagcaatgggcagccggagaacaactacaagaccacgcctcccgtgctggactccgacggctccttcttcctctatagcaagctcaccgtggacaagagcaggtggcagcaggggaacgtcttctcatgctccgtgatgcatgaggctctgcacaaccactacacgcagaagagcttaagcctgtctccgggtaaatga

SEQ ID NO: 128 - DNA, 1353 bp, Artificial Sequence
  Antibody z13 Heavy Chain DNA Sequences
caggtgcagctggtgcagagcggagccgaagtgaagaagcccggcgccagcgtgaaggtgagctgcaaggccagcggctacaccttcaccaactacggcatgaactgggtgagacaggcccctggacagggactggagtggatgggctggatcaacacctacaccggcgagcccacctacgccgacgacttcaagggcagggtgaccttcaccctggacaccagcaccagcaccgcctacatggagctgaggagcctgaggagcgacgacatggccgtgtactattgcgccaggaagagcaccgtggtgagcaggtacttcgacgtgtggggccagggaaccaccgtgaccgtgagcagcgcgtcgaccaagggcccatccgtcttccccctggcaccctcctccaagagcacctctgggggcacagcggccctgggctgcctggtcaaggactacttccccgaaccggtgacggtgtcctggaactcaggcgctctgaccagcggcgtgcacaccttcccggctgtcctacagtcctcaggactctactccctcagcagcgtggtgaccgtgccctccagcagcttgggcacccagacctacatctgcaacgtgaatcacaagcccagcaacaccaaggtggacaagagagttgagcccaaatcttgtgacaaaactcacacatgcccaccgtgcccagcacctgaactcctggggggaccgtcagtcttcctcttccccccaaaacccaaggacaccctcatgatctcccggacccctgaggtcacatgcgtggtggtggacgtgagccacgaagaccctgaggtcaagttcaactggtacgtggacggcgtggaggtgcataatgccaagacaaagccgcgggaggagcagtacaacagcacgtaccgtgtggtcagcgtcctcaccgtcctgcaccaggactggctgaatggcaaggagtacaagtgcaaggtctccaacaaagccctcccagcccccatcgagaaaaccatctccaaagccaaagggcagccccgagaaccacaggtctacaccctgcccccatcccgggaggagatgaccaagaaccaggtcagcctgacctgcctggtcaaaggcttctatcccagcgacatcgccgtggagtgggagagcaatgggcagccggagaacaactacaagaccacgcctcccgtgctggactccgacggctccttcttcctctatagcaagctcaccgtggacaagagcaggtggcagcaggggaacgtcttctcatgctccgtgatgcatgaggctctgcacaaccactacacgcagaagagcttaagcctgtctccgggtaaatga

SEQ ID NO: 129 - DNA, 1353 bp, Artificial Sequence
  Antibody xAb Heavy Chain DNA Sequences
cagatccagttggtgcagtctggacctgagctgaagaagcctggagagacagtcaagatctcctgcaaggcttctggatataccttcacaaactatggaatgaactgggtgaagcaggctccaggaaagggtttaaagtggatgggctggataaacacctacactggagagccaacatatgctgatgacttcaagggacggtttgtcttctctttggaaacctctgccagcactgcctacttgcagatcaacaacctcaaaaatgaggacatggccacatatttctgtgcaagaaaaagtacggtagtaagtaggtacttcgatgtctggggcgcagggaccacggtcaccgtctcctcagcgtcgaccaagggcccatccgtcttccccctggcaccctcctccaagagcacctctgggggcacagcggccctgggctgcctggtcaaggactacttccccgaaccggtgacggtgtcctggaactcaggcgctctgaccagcggcgtgcacaccttcccggctgtcctacagtcctcaggactctactccctcagcagcgtggtgaccgtgccctccagcagcttgggcacccagacctacatctgcaacgtgaatcacaagcccagcaacaccaaggtggacaagagagttgagcccaaatcttgtgacaaaactcacacatgcccaccgtgcccagcacctgaactcctggggggaccgtcagtcttcctcttccccccaaaacccaaggacaccctcatgatctcccggacccctgaggtcacatgcgtggtggtggacgtgagccacgaagaccctgaggtcaagttcaactggtacgtggacggcgtggaggtgcataatgccaagacaaagccgcgggaggagcagtacaacagcacgtaccgtgtggtcagcgtcctcaccgtcctgcaccaggactggctgaatggcaaggagtacaagtgcaaggtctccaacaaagccctcccagcccccatcgagaaaaccatctccaaagccaaagggcagccccgagaaccacaggtctacaccctgcccccatcccgggaggagatgaccaagaaccaggtcagcctgacctgcctggtcaaaggcttctatcccagcgacatcgccgtggagtgggagagcaatgggcagccggagaacaactacaagaccacgcctcccgtgctggactccgacggctccttcttcctctatagcaagctcaccgtggacaagagcaggtggcagcaggggaacgtcttctcatgctccgtgatgcatgaggctctgcacaaccactacacgcagaagagcttaagcctgtctccgggtaaatga

SEQ ID NO: 130 - DNA, 645 bp, Artificial Sequence
  Antibody xAb Light Chain DNA Sequences
gacattgtgctgacccagtctcacaaattcatgtccacatcagtaggagacagggtcagcatcacctgcaaggccagtcaggatgtgggtgatgctgtaacctggtgtcaacagaaaccaggtcaacctcctaaactactgatttactgggcatccacccggcacactggagtccctgatcgcttcacaggcagtgggtctgggacagatttcactctcaccattaacaatgtgcagtctgaggacttggcagattatttctgtcagcaatatcgcagctatcctctcacgttcggtgctgggaccaagctggagctgaaacgtacggtggctgcaccatctgtcttcatcttcccgccatctgatgagcagttgaaatctggaactgcctctgttgtgtgcctgctgaataacttctatcccagagaggccaaagtacagtggaaggtggataacgccctccaatcgggtaactcccaggagagtgtcacagagcaggacagcaaggacagcacctacagcctcagcagcaccctgacgctgagcaaagcagactacgagaaacacaaagtctacgcctgcgaagtcacccatcagggcctgagctcgcccgtcacaaagagcttcaacaggggagagtgttga

SEQ ID NO: 131 - protein, 999 aa, Homo sapiens
  Full-Length Human MERTK (Swiss-Prot ID: Q12866.2)
MGPAPLPLLLGLFLPALWRRAITEAREEAKPYPLFPGPFPGSLQTDHTPLLSLPHASGYQPALMFSPTQPGRPHTGNVAIPQVTSVESKPLPPLAFKHTVGHIILSEHKGVKFNCSISVPNIYQDTTISWWKDGKELLGAHHAITQFYPDDEVTAIIASFSITSVQRSDNGSYICKMKINNEEIVSDPIYIEVQGLPHFTKQPESMNVTRNTAFNLTCQAVGPPEPVNIFWVQNSSRVNEQPEKSPSVLTVPGLTEMAVFSCEAHNDKGLTVSKGVQINIKAIPSPPTEVSIRNSTAHSILISWVPGFDGYSPFRNCSIQVKEADPLSNGSVMIFNTSALPHLYQIKQLQALANYSIGVSCMNEIGWSAVSPWILASTTEGAPSVAPLNVTVFLNESSDNVDIRWMKPPTKQQDGELVGYRISHVWQSAGISKELLEEVGQNGSRARISVQVHNATCTVRIAAVTRGGVGPFSDPVKIFIPAHGWVDYAPSSTPAPGNADPVLIIFGCFCGFILIGLILYISLAIRKRVQETKFGNAFTEEDSELVVNYIAKKSFCRRAIELTLHSLGVSEELQNKLEDVVIDRNLLILGKILGEGEFGSVMEGNLKQEDGTSLKVAVKTMKLDNSSQREIEEFLSEAACMKDFSHPNVIRLLGVCIEMSSQGIPKPMVILPFMKYGDLHTYLLYSRLETGPKHIPLQTLLKFMVDIALGMEYLSNRNFLHRDLAARNCMLRDDMTVCVADFGLSKKIYSGDYYRQGRIAKMPVKWIAIESLADRVYTSKSDVWAFGVTMWEIATRGMTPYPGVQNHEMYDYLLHGHRLKQPEDCLDELYEIMYSCWRTDPLDRPTFSVLRLQLEKLLESLPDVRNQADVIYVNTQLLESSEGLAQGSTLAPLDLNIDPDSIIASCTPRAAISVVTAEVHDSKPHEGRYILNGGSEEWEDLTSAPSAAVTAEKNSVLPGERLVRNGVSWSHSSMLPLGSSLPDELLFADDSSEGSEVLM

SEQ ID NO: 132 - protein, 474 aa, Artificial Sequence
  Extracellular Doman of MERTK Used for Immunization
REEAKPYPLFPGPFPGSLQTDHTPLLSLPHASGYQPALMFSPTQPGRPHTGNVAIPQVTSVESKPLPPLAFKHTVGHIILSEHKGVKFNCSISVPNIYQDTTISWWKDGKELLGAHHAITQFYPDDEVTAIIASFSITSVQRSDNGSYICKMKINNEEIVSDPIYIEVQGLPHFTKQPESMNVTRNTAFNLTCQAVGPPEPVNIFWVQNSSRVNEQPEKSPSVLTVPGLTEMAVFSCEAHNDKGLTVSKGVQINIKAIPSPPTEVSIRNSTAHSILISWVPGFDGYSPFRNCSIQVKEADPLSNGSVMIFNTSALPHLYQIKQLQALANYSIGVSCMNEIGWSAVSPWILASTTEGAPSVAPLNVTVFLNESSDNVDIRWMKPPTKQQDGELVGYRISHVWQSAGISKELLEEVGQNGSRARISVQVHNATCTVRIAAVTRGGVGPFSDPVKIFIPAHGWVDYAPSSTPAPGNA